European Patent Application EP 4 556 905 A1, published May 21, 2025. Title: Method for the screening of active agents that inhibit changes in the structure of a transcription factor comprising amino acid repeat mutations. Applicant: Consejo Superior de Investigaciones Cientificas (CSIC). The sequence listing filed with the application follows.

SEQUENCE LISTING (23 sequences)

SEQ ID NO: 1 - DNA, 34 bp, synthetic construct
  source 1..34: mol_type = other DNA; note = Primer forward XL20 insert; note (original language) = Cebafor directo XL20 inserto; organism (original language) = construccion sintetica
atttccagggatccatgtataaaatggaatattc

SEQ ID NO: 2 - DNA, 28 bp, synthetic construct
  source 1..28: mol_type = other DNA; note = Primer reverse XL20 insert; note (original language) = Cebador reverso XL20 inserto; organism (original language) = construccion sintetica
gtggtgctcgagttagaacatactgctc

SEQ ID NO: 3 - DNA, 23 bp, synthetic construct
  source 1..23: mol_type = other DNA; note = Primer forward XL20 vector; note (original language) = Cebador directo XL20 vector; organism (original language) = construccion sintetica
ctcgagcaccaccaccaccactg

SEQ ID NO: 4 - DNA, 29 bp, synthetic construct
  source 1..29: mol_type = other DNA; note = Primer reverse XL20 vector; note (original language) = Cebador reverso XL20 vector; organism (original language) = construccion sintetica
gacatggatccctggaaatacaggttttc

SEQ ID NO: 5 - DNA, 31 bp, synthetic construct
  source 1..31: mol_type = other DNA; note = Primer forward L20 insert; note (original language) = Cebador directo L20 inserto; organism (original language) = construccion sintetica
atttccagggatccatccgcaccaccttcac

SEQ ID NO: 6 - DNA, 28 bp, synthetic construct
  source 1..28: mol_type = other DNA; note = Primer reverse L20 insert; note (original language) = Cebador reverso L20 inserto; organism (original language) = consutrccion sintetica
gtggtgctcgagttagaacatactgctc

SEQ ID NO: 7 - DNA, 30 bp, synthetic construct
  source 1..30: mol_type = other DNA; note = Primer forward S20 insert; note (original language) = Cebador directo S20 inserto; organism (original language) = consturccion sintetica
atttccagggatccgctaagtttcgcaagc

SEQ ID NO: 8 - DNA, 28 bp, synthetic construct
  source 1..28: mol_type = other DNA; note = Primer revers S20 insert; note (original language) = Cebador reverso S20 insert; organism (original language) = construccion sintetica
gtggtgctcgagttagaacatactgctc

SEQ ID NO: 9 - DNA, 30 bp, synthetic construct
  source 1..30: mol_type = other DNA; note = Primer reverse S20 vector; note (original language) = Cebador reverso S20 vector; organism (original language) = consturccion sintetica
cttagcggatccctggaaatacaggttttc

SEQ ID NO: 10 - DNA, 31 bp, synthetic construct
  source 1..31: mol_type = other DNA; note = Primer forward XS20 insert; note (original language) = Cebador directo XS20 inserto; organism (original language) = construccion sintetica
atttccagggatccggcccggggggcccggg

SEQ ID NO: 11 - DNA, 28 bp, synthetic construct
  source 1..28: mol_type = other DNA; note = Primer reverse XS20 insert; note (original language) = Cebador reverso XS20 inserto; organism (original language) = construccion sintetica
gtggtgctcgagttagaacatactgctc

SEQ ID NO: 12 - DNA, 23 bp, synthetic construct
  source 1..23: mol_type = other DNA; note = Primer forward XS20 vector; note (original language) = Cebador directo XS20 vector; organism (original language) = construccion sintetica
ctcgagcaccaccaccaccactg

SEQ ID NO: 13 - DNA, 29 bp, synthetic construct
  source 1..29: mol_type = other DNA; note = Primer reverse XS20 vector; note (original language) = Cebador reverso XS20 vector; organism (original language) = construccion sintetica
gggccggatccctggaaatacaggttttc

SEQ ID NO: 14 - DNA, 33 bp, synthetic construct
  source 1..33: mol_type = other DNA; note = Primer forward XS23; note (original language) = Cebador directo XS23; organism (original language) = construccion sintetica
gcaagggcggtgcagcagcagcggctgcggctg

SEQ ID NO: 15 - DNA, 33 bp, synthetic construct
  source 1..33: mol_type = other DNA; note = Primer reverse XS23; note (original language) = Cebador reverso XS23; organism (original language) = construccion sintetica
cagccgcagccgctgctgctgcaccgcccttgc

SEQ ID NO: 16 - DNA, 32 bp, synthetic construct
  source 1..32: mol_type = other DNA; note = Primer reverse XS26; note (original language) = Cebador reverso XS26; organism (original language) = construccion sintetica
cgctgctgctgctgctgcagcaccgcccttgc

SEQ ID NO: 17 - DNA, 32 bp, synthetic construct
  source 1..32: mol_type = other DNA; note = Primer reverse C315; note (original language) = Cebador reverso C315; organism (original language) = construccion sintetica
ggtggtgctcgagttaacagaacatactgctc

SEQ ID NO: 18 - protein, 87 aa, synthetic construct
  source 1..87: note = Human PHOX2B transcription factor fragment comprising 20 alanine residues (XS20); note (original language) = Fragmento del factor de transcripción PHOX2B humano que comprende 20 residuos de alanina (XS20); organism (original language) = construccion sintetica
GPGGPGGEPGKGGAAAAAAAAAAAAAAAAAAAAGGLAAAGGPGQGWAPGPGPITSIPDSLGGPFASVLSSLQRPNGAKAALVKSSMF

SEQ ID NO: 19 - protein, 90 aa, synthetic construct
  source 1..90: note = Human PHOX2B transcription factor fragment comprising 23 alanine residues (XS23); note (original language) = Fragmento del factor de transcripción humano PHOX2B que comprende 23 residuos de alanina (XS23); organism (original language) = construccion sintetica
GPGGPGGEPGKGGAAAAAAAAAAAAAAAAAAAAAAAGGLAAAGGPGQGWAPGPGPITSIPDSLGGPFASVLSSLQRPNGAKAALVKSSMF

SEQ ID NO: 20 - protein, 93 aa, synthetic construct
  source 1..93: note = Human PHOX2B transcription factor fragment comprising 26 alanine residues (XS26); note (original language) = Fragmento del factor de transcripción humano PHOX2B que comrpende 26 residuos de alanina (XS26); organism (original language) = construccion sintetica
GPGGPGGEPGKGGAAAAAAAAAAAAAAAAAAAAAAAAAAGGLAAAGGPGQGWAPGPGPITSIPDSLGGPFASVLSSLQRPNGAKAALVKSSMF

SEQ ID NO: 21 - DNA, 23 bp, synthetic construct
  source 1..23: mol_type = other DNA; note = Primer forward S20 vector; note (original language) = Cebador directo S20 vector; organism (original language) = construccion sintetica
ctcgagcaccaccaccaccactg

SEQ ID NO: 22 - DNA, 32 bp, synthetic construct
  source 1..32: mol_type = other DNA; note = Primer forward XS26; note (original language) = Cebador directo XS26; organism (original language) = construccion sintetica
gcaagggcggtgctgcagcagcagcagcagcg

SEQ ID NO: 23 - DNA, 32 bp, synthetic construct
  source 1..32: mol_type = other DNA; note = Primer forward C315; note (original language) = Cebador directo C315; organism (original language) = construccion sintetica
gagcagtatgttctgttaactcgagcaccacc